European Patent Specification EP 3 899 051 B1, published April 3, 2024. Title: ASSAY FOR DETECTING HUMAN PAPILLOMA VIRUS (HPV). Applicant: ABBOTT MOLECULAR INC. The sequence listing filed with the application follows.

SEQUENCE LISTING (32 sequences)

SEQ ID NO: 1 - DNA, 25 bp, Artificial sequence
  Synthetic
tatttgttactgtggtagatactac

SEQ ID NO: 2 - DNA, 29 bp, Artificial sequence
  Synthetic
caattgtttgttactgttgtggatactac

SEQ ID NO: 3 - DNA, 25 bp, Artificial sequence
  Synthetic
tttttattacctgtgttgatactac

SEQ ID NO: 4 - DNA, 25 bp, Artificial sequence
  Synthetic
tatttgttactgttgttgatactac

SEQ ID NO: 5 - DNA, 28 bp, Artificial sequence
  Synthetic
gaaaaataaactgtaaatcatattcctc

SEQ ID NO: 6 - DNA, 35 bp, Artificial sequence
  Synthetic
tgaaaaataaactgtaaatcatattcttcaccatg

SEQ ID NO: 7 - DNA, 20 bp, Artificial sequence
  Synthetic
ctgccatatctacttcagaa

SEQ ID NO: 8 - DNA, 22 bp, Artificial sequence
  Synthetic
cacagtctcctgtacctgggca

SEQ ID NO: 9 - DNA, 20 bp, Artificial sequence
  Synthetic
aagtagtaattttaaagagt

SEQ ID NO: 10 - DNA, 19 bp, Artificial sequence
  Synthetic
atgcacacaagtaactagt

SEQ ID NO: 11 - DNA, 22 bp, Artificial sequence
  Synthetic
cctactaagtttaagcagtata

SEQ ID NO: 12 - DNA, 14 bp, Artificial sequence
  Synthetic
aaaaaggaaagcac

SEQ ID NO: 13 - DNA, 19 bp, Artificial sequence
  Synthetic
tgacattatgcactgaagt

SEQ ID NO: 14 - DNA, 19 bp, Artificial sequence
  Synthetic
ctgtgtgttctgctgtgtc

SEQ ID NO: 15 - DNA, 14 bp, Artificial sequence
  Synthetic
tccataccttctac

SEQ ID NO: 16 - DNA, 19 bp, Artificial sequence
  Synthetic
ttagcactgccactgctgc

SEQ ID NO: 17 - DNA, 19 bp, Artificial sequence
  Synthetic
ttacttaactgttctgtag

SEQ ID NO: 18 - DNA, 24 bp, Artificial sequence
  Synthetic
attcctaatgtatacacacctacc

SEQ ID NO: 19 - DNA, 22 bp, Artificial sequence
  Synthetic
caatcaataccttcgccatgtg

SEQ ID NO: 20 - DNA, 19 bp, Artificial sequence
  Synthetic
ctttgtctactactactga

SEQ ID NO: 21 - DNA, 19 bp, Artificial sequence
  Synthetic
cattgtccactactacaga

SEQ ID NO: 22 - DNA, 17 bp, Artificial sequence
  Synthetic
gttggtatcaaggttac

SEQ ID NO: 23 - DNA, 22 bp, Artificial sequence
  Synthetic
cctaagggtgggaaaatagacc

SEQ ID NO: 24 - DNA, 28 bp, Artificial sequence
  Synthetic
tttctgataggcactgactctctctgcc

SEQ ID NO: 25 - DNA, 20 bp, Artificial sequence
  Synthetic
  misc_feature (1)..(1): pdC (propyne modified C)
  misc_feature (2)..(2): pdU (propyne modified T)
  misc_feature (4)..(5): pdC (propyne modified C)
  misc_feature (7)..(7): pdU (propyne modified T)
  misc_feature (9)..(9): pdU (propyne modified T)
  misc_feature (10)..(10): pdC (propyne modified C)
  misc_feature (11)..(11): pdU (propyne modified T)
  misc_feature (13)..(13): pdC (propyne modified C)
  misc_feature (14)..(15): pdU (propyne modified T)
ctgccatatctacttcagaa

SEQ ID NO: 26 - DNA, 20 bp, Artificial sequence
  Synthetic
  misc_feature (4)..(4): pdU (propyne modified T)
  misc_feature (7)..(7): pdU (propyne modified T)
  misc_feature (10)..(13): pdU (propyne modified T)
  misc_feature (20)..(20): pdU (propyne modified T)
aagtagtaattttaaagagt

SEQ ID NO: 27 - DNA, 19 bp, Artificial sequence
  Synthetic
  misc_feature (2)..(2): pdU (propyne modified T)
  misc_feature (4)..(4): pdC (propyne modified C)
  misc_feature (6)..(6): pdC (propyne modified C)
  misc_feature (8)..(8): pdC (propyne modified C)
  misc_feature (12)..(12): pdU (propyne modified T)
  misc_feature (15)..(15): pdC (propyne modified C)
  misc_feature (16)..(16): pdU (propyne modified T)
  misc_feature (19)..(19): pdU (propyne modified T)
atgcacacaagtaactagt

SEQ ID NO: 28 - DNA, 14 bp, Artificial sequence
  Synthetic
  misc_feature (12)..(12): pdC (propyne modified C)
  misc_feature (14)..(14): pdC (propyne modified C)
aaaaaggaaagcac

SEQ ID NO: 29 - DNA, 19 bp, Artificial sequence
  Synthetic
  misc_feature (1)..(1): pdU (propyne modified T)
  misc_feature (4)..(4): pdC (propyne modified C)
  misc_feature (6)..(7): pdU (propyne modified T)
  misc_feature (9)..(9): pdU (propyne modified T)
  misc_feature (11)..(11): pdC (propyne modified C)
  misc_feature (13)..(13): pdC (propyne modified C)
  misc_feature (14)..(14): pdU (propyne modified T)
  misc_feature (19)..(19): pdU (propyne modified T)
tgacattatgcactgaagt

SEQ ID NO: 30 - DNA, 14 bp, Artificial sequence
  Synthetic
  misc_feature (1)..(1): pdU (propyne modified T)
  misc_feature (2)..(3): pdC (propyne modified C)
  misc_feature (5)..(5): pdU (propyne modified T)
  misc_feature (7)..(8): pdC (propyne modified C)
  misc_feature (9)..(10): pdU (propyne modified T)
  misc_feature (11)..(11): pdC (propyne modified C)
  misc_feature (12)..(12): pdU (propyne modified T)
  misc_feature (14)..(14): pdC (propyne modified C)
tccataccttctac

SEQ ID NO: 31 - DNA, 19 bp, Artificial sequence
  Synthetic
  misc_feature (1)..(2): pdU (propyne modified T)
  misc_feature (5)..(5): pdC (propyne modified C)
  misc_feature (7)..(7): pdC (propyne modified C)
  misc_feature (8)..(8): pdU (propyne modified T)
  misc_feature (10)..(10): pdC (propyne modified C)
  misc_feature (13)..(13): pdC (propyne modified C)
  misc_feature (14)..(14): pdU (propyne modified T)
  misc_feature (16)..(16): pdC (propyne modified C)
  misc_feature (17)..(17): pdU (propyne modified T)
  misc_feature (19)..(19): pdC (propyne modified C)
ttagcactgccactgctgc

SEQ ID NO: 32 - DNA, 19 bp, Artificial sequence
  Synthetic
  misc_feature (1)..(2): pdU (propyne modified T)
  misc_feature (4)..(4): pdC (propyne modified C)
  misc_feature (5)..(6): pdU (propyne modified T
  misc_feature (9)..(9): pdC (propyne modified C)
  misc_feature (10)..(10): pdU (propyne modified T
  misc_feature (12)..(13): pdU (propyne modified T
  misc_feature (14)..(14): pdC (propyne modified C)
  misc_feature (15)..(15): pdU (propyne modified T)
  misc_feature (17)..(17): pdU (propyne modified T)
ttacttaactgttctgtag